European Patent Specification EP 3 775 146 B1, published March 4, 2026. Title: PROCESS FOR THE PREPARATION OF A STABLE BEVERAGE. Applicant: DSM IP Assets B.V. The sequence listing filed with the application follows.

SEQUENCE LISTING (2 sequences)

SEQ ID NO: 1 - protein, 640 aa, Fusarium graminearum
MHLLNGKTAAVALALLNSCNALKVTILADTNRDGKVDNNDINGKSTWTNNRGALILPNIGDTGSRCAKQWGPSVDIQGDESYLDKCNDASDNVQRNPKYLASLKTLPLTTLSATAKGSIIIADKTGASKVRIFVKQSGKWNYVAADHVFTAKELKSGLELGVDARDVRRPQDWNGYAKIQFTVTDGKTKATDAVAVRVAPVLTHHHGQHAQRIFTTGVNEAGVNKVQETFIADILRNVAGAGIKEPVFQFHNQDIWTQDFFEPGYASIPGPNGPVSIRIMIRSAQSSRRSGRDAFHDLRNDQVGAVQHPGDGDSIDSTGNLETIPPYSHNGKSFPVGRTIMGAWDGRAPLMVEFLKAQQVQEPLILDTSWLYVGHVDEFIQFLPSNNKLGWVIMVADPMKGVDLLKKAVKTGHGKVKAVSRPLSADEKKEQLCLPRQTIAEALKFKSFDAINKHSAERIQANLDIIKRETGITDEDIHRVPALFYYTQSNSWLCPGETAEDDSAQPQKAASNSGITMKTSQGGPGFKAKSIVEAATPGKSIQRRVIDPATQVTALYPGSVNGLVMTDTKILAPSPWGPVINKQDIFAAAVSQVYTNAGYNVTYQDDWFSHFKLQGDVHCGSNSWREIPKKWWDSLRVNNY

SEQ ID NO: 2 - protein, 521 aa, Artificial Sequence
  Protein sequence of A. niger proline-specific endoprotease with pectinemethylesterease signal sequence
MVKSILASVFFAATALAARPRLVPKPVSRPASSKSAATTGEAYFEQLLDHHNPEKGTFSQRYWWSTEYWGGPGSPVVLFTPGEVSADGYEGYLTNETLTGVYAQEIQGAVILIEHRYWGDSSPYEVLNAETLQYLTLDQAILDMTYFAETVKLQFDNSTRSNAQNAPWVMVGGSYSGALTAWTESVAPGTFWAYHATSAPVEAIYDYWQYFYPIQQGMAQNCSKDVSLVAEYVDKIGKNGTAKEQQALKELFGLGAVEHFDDFAAVLPNGPYLWQDNDFATGYSSFFQFCDAVEGVEAGAAVTPGPEGVGLEKALANYANWFNSTILPDYCASYGYWTDEWSVACFDSYNASSPIYTDTSVGNAVDRQWEWFLCNEPFFYWQDGAPEGTSTIVPRLVSASYWQRQCPLYFPETNGYTYGSAKGKNAATVNSWTGGWDMTRNTTRLIWTNGQYDPWRDSGVSSTFRPGGPLASTANEPVQIIPGGFHCSDLYMADYYANEGVKKVVDNEVKQIKEWVEEYYA